European Patent Application EP 4 778 529 A1, published July 22, 2026. Title: 心筋再生、心筋線維化の抑制または心疾患の処置用の医薬組成物. Applicant: Kyoto University. The sequence listing filed with the application follows.

SEQUENCE LISTING (11 sequences)

SEQ ID NO: 1 - protein, 756 aa, Homo sapiens
MSWSPSLTTQTCGAWEMKERLGTGGFGNVIRWHNQETGEQIAIKQCRQELSPRNRERWCLEIQIMRRLTHPNVVAARDVPEGMQNLAPNDLPLLAMEYCQGGDLRKYLNQFENCCGLREGAILTLLSDIASALRYLHENRIIHRDLKPENIVLQQGEQRLIHKIIDLGYAKELDQGSLCTSFVGTLQYLAPELLEQQKYTVTVDYWSFGTLAFECITGFRPFLPNWQPVQWHSKVRQKSEVDIVVSEDLNGTVKFSSSLPYPNNLNSVLAERLEKWLQLMLMWHPRQRGTDPTYGPNGCFKALDDILNLKLVHILNMVTGTIHTYPVTEDESLQSLKARIQQDTGIPEEDQELLQEAGLALIPDKPATQCISDGKLNEGHTLDMDLVFLFDNSKITYETQISPRPQPESVSCILQEPKRNLAFFQLRKVWGQVWHSIQTLKEDCNRLQQGQRAAMMNLLRNNSCLSKMKNSMASMSQQLKAKLDFFKTSIQIDLEKYSEQTEFGITSDKLLLAWREMEQAVELCGRENEVKLLVERMMALQTDIVDLQRSPMGRKQGGTLDDLEEQARELYRRLREKPRDQRTEGDSQEMVRLLLQAIQSFEKKVRVIYTQLSKTVVCKQKALELLPKVEEVVSLMNEDEKTVVRLQEKRQKELWNLLKIACSKVRGPVSGSPDSMNASRLSQPGQLMSQPSTASNSLPEPAKKSEELVAEAHNLCTLLENAIQDTVREQDQSFTALDWSWLQTEEEEHSCLEQAS

SEQ ID NO: 2 - protein, 757 aa, Mus musculus
MSWSPSLPTQTCGAWEMKERLGTGGFGNVIRWHNQATGEQIAIKQCRQELSPKNRDRWCLEIQIMRRLNHPNVVAARDVPEGMQNLAPNDLPLLAMEYCQGGDLRRYLNQFENCCGLREGAVLTLLSDIASALRYLHENRIIHRDLKPENIVLQQGEKRLIHKIIDLGYAKELDQGSLCTSFVGTLQYLAPELLEQQKYTVTVDYWSFGTLAFECITGFRPFLPNWQPVQWHSKVRQKSEVDIVVSEDLNGAVKFSSSLPFPNNLNSVLAERLEKWLQLMLMWHPRQRGTDPQYGPNGCFRALDDILNLKLVHVLNMVTGTVHTYPVTEDESLQSLKTRIQEDTGILETDQELLQEAGLVLLPDKPATQCISDSKTNEGLTLDMDLVFLFDNSKINYETQITPRPQPESVSCILQEPKRNLSFFQLRKVWGQVWHSIQTLKEDCNRLQQGQRAAMMSLLRNNSCLSKMKNAMASTAQQLKAKLDFFKTSIQIDLEKYKEQTEFGITSDKLLLAWREMEQAVEQCGRENDVKHLVERMMALQTDIVDLQRSPMGRKQGGTLDDLEEQARELYRRLREKPRDQRTEGDSQEMVRLLLQAIQSFEKKVRVIYTQLSKTVVCKQKALELLPKVEEVVSLMNEDERTVVRLQEKRQKELWNLLKIACSKVRGPVSGSPDSMNVSRLSHPGQLMSQPSSACDSLPESDKKSEELVAEAHALCSRLESALQDTVKEQDRSFTTLDWSWLQMEDEERCSLEQACD

SEQ ID NO: 3 - protein, 756 aa, Homo sapiens
MSWSPSLTTQTCGAWEMKERLGTGGFGNVIRWHNQETGEQIAIKQCRQELSPRNRERWCLEIQIMRRLTHPNVVAARDVPEGMQNLAPNDLPLLAMEYCQGGDLRKYLNQFENCCGLREGAILTLLSDIASALRYLHENRIIHRDLKPENIVLQQGEQRLIHKIIDLGYAKELDQGELCTEFVGTLQYLAPELLEQQKYTVTVDYWSFGTLAFECITGFRPFLPNWQPVQWHSKVRQKSEVDIVVSEDLNGTVKFSSSLPYPNNLNSVLAERLEKWLQLMLMWHPRQRGTDPTYGPNGCFKALDDILNLKLVHILNMVTGTIHTYPVTEDESLQSLKARIQQDTGIPEEDQELLQEAGLALIPDKPATQCISDGKLNEGHTLDMDLVFLFDNSKITYETQISPRPQPESVSCILQEPKRNLAFFQLRKVWGQVWHSIQTLKEDCNRLQQGQRAAMMNLLRNNSCLSKMKNSMASMSQQLKAKLDFFKTSIQIDLEKYSEQTEFGITSDKLLLAWREMEQAVELCGRENEVKLLVERMMALQTDIVDLQRSPMGRKQGGTLDDLEEQARELYRRLREKPRDQRTEGDSQEMVRLLLQAIQSFEKKVRVIYTQLSKTVVCKQKALELLPKVEEVVSLMNEDEKTVVRLQEKRQKELWNLLKIACSKVRGPVSGSPDSMNASRLSQPGQLMSQPSTASNSLPEPAKKSEELVAEAHNLCTLLENAIQDTVREQDQSFTALDWSWLQTEEEEHSCLEQAS

SEQ ID NO: 4 - protein, 757 aa, Mus musculus
MSWSPSLPTQTCGAWEMKERLGTGGFGNVIRWHNQATGEQIAIKQCRQELSPKNRDRWCLEIQIMRRLNHPNVVAARDVPEGMQNLAPNDLPLLAMEYCQGGDLRRYLNQFENCCGLREGAVLTLLSDIASALRYLHENRIIHRDLKPENIVLQQGEKRLIHKIIDLGYAKELDQGELCTEFVGTLQYLAPELLEQQKYTVTVDYWSFGTLAFECITGFRPFLPNWQPVQWHSKVRQKSEVDIVVSEDLNGAVKFSSSLPFPNNLNSVLAERLEKWLQLMLMWHPRQRGTDPQYGPNGCFRALDDILNLKLVHVLNMVTGTVHTYPVTEDESLQSLKTRIQEDTGILETDQELLQEAGLVLLPDKPATQCISDSKTNEGLTLDMDLVFLFDNSKINYETQITPRPQPESVSCILQEPKRNLSFFQLRKVWGQVWHSIQTLKEDCNRLQQGQRAAMMSLLRNNSCLSKMKNAMASTAQQLKAKLDFFKTSIQIDLEKYKEQTEFGITSDKLLLAWREMEQAVEQCGRENDVKHLVERMMALQTDIVDLQRSPMGRKQGGTLDDLEEQARELYRRLREKPRDQRTEGDSQEMVRLLLQAIQSFEKKVRVIYTQLSKTVVCKQKALELLPKVEEVVSLMNEDERTVVRLQEKRQKELWNLLKIACSKVRGPVSGSPDSMNVSRLSHPGQLMSQPSSACDSLPESDKKSEELVAEAHALCSRLESALQDTVKEQDRSFTTLDWSWLQMEDEERCSLEQACD

SEQ ID NO: 5 - DNA, 2268 bp, Homo sapiens
  source 1..2268: mol_type = genomic DNA
atgagctggtcaccttccctgacaacgcagacatgtggggcctgggaaatgaaagagcgccttgggacagggggatttggaaatgtcatccgatggcacaatcaggaaacaggtgagcagattgccatcaagcagtgccggcaggagctcagcccccggaaccgagagcggtggtgcctggagatccagatcatgagaaggctgacccaccccaatgtggtggctgcccgagatgtccctgaggggatgcagaacttggcgcccaatgacctgcccctgctggccatggagtactgccaaggaggagatctccggaagtacctgaaccagtttgagaactgctgtggtctgcgggaaggtgccatcctcaccttgctgagtgacattgcctctgcgcttagataccttcatgaaaacagaatcatccatcgggatctaaagccagaaaacatcgtcctgcagcaaggagaacagaggttaatacacaaaattattgacctaggatatgccaaggagctggatcagggcgaactttgcacagaattcgtggggaccctgcagtacctggccccagagctactggagcagcagaagtacacagtgaccgtcgactactggagcttcggcaccctggcctttgagtgcatcacgggcttccggcccttcctccccaactggcagcccgtgcagtggcattcaaaagtgcggcagaagagtgaggtggacattgttgttagcgaagacttgaatggaacggtgaagttttcaagctctttaccctaccccaataatcttaacagtgtcctggctgagcgactggagaagtggctgcaactgatgctgatgtggcacccccgacagaggggcacggatcccacgtatgggcccaatggctgcttcaaggccctggatgacatcttaaacttaaagttggttcatatcttgaacatggtcacgggcaccatccacacctaccctgtgacagaggatgagagtctgcagagcttgaaggccagaatccaacaggacacgggcatcccagaggaggaccaggagctgctgcaggaagcgggcctggcgttgatccccgataagcctgccactcagtgtatttcagacggcaagttaaatgagggccacacattggacatggatcttgtttttctctttgacaacagtaaaatcacctatgagactcagatctccccacggccccaacctgaaagtgtcagctgtatccttcaagagcccaagaggaatctcgccttcttccagctgaggaaggtgtggggccaggtctggcacagcatccagaccctgaaggaagattgcaaccggctgcagcagggacagcgagccgccatgatgaatctcctccgaaacaacagctgcctctccaaaatgaagaattccatggcttccatgtctcagcagctcaaggccaagttggatttcttcaaaaccagcatccagattgacctggagaagtacagcgagcaaaccgagtttgggatcacatcagataaactgctgctggcctggagggaaatggagcaggctgtggagctctgtgggcgggagaacgaagtgaaactcctggtagaacggatgatggctctgcagaccgacattgtggacttacagaggagccccatgggccggaagcaggggggaacgctggacgacctagaggagcaagcaagggagctgtacaggagactaagggaaaaacctcgagaccagcgaactgagggtgacagtcaggaaatggtacggctgctgcttcaggcaattcagagcttcgagaagaaagtgcgagtgatctatacgcagctcagtaaaactgtggtttgcaagcagaaggcgctggaactgttgcccaaggtggaagaggtggtgagcttaatgaatgaggatgagaagactgttgtccggctgcaggagaagcggcagaaggagctctggaatctcctgaagattgcttgtagcaaggtccgtggtcctgtcagtggaagcccggatagcatgaatgcctctcgacttagccagcctgggcagctgatgtctcagccctccacggcctccaacagcttacctgagccagccaagaagagtgaagaactggtggctgaagcacataacctctgcaccctgctagaaaatgccatacaggacactgtgagggaacaagaccagagtttcacggccctagactggagctggttacagacggaagaagaagagcacagctgcctggagcaggcctca

SEQ ID NO: 6 - DNA, 2271 bp, Mus musculus
  source 1..2271: mol_type = genomic DNA
atgagctggtcaccgtccctcccaacccagacatgtggagcctgggaaatgaaagaacgcctggggaccgggggatttggaaacgtcatccggtggcacaatcaggcgacaggtgaacagatcgccatcaagcaatgccgacaggagctcagcccaaagaacagagaccgctggtgcctcgaaatccagatcatgagaaggctgaaccatcccaatgtggtggctgcccgggatgtcccagaggggatgcagaacctggcacccaatgatttgccactgctggccatggagtactgccaaggaggagatctccgaagatacttgaaccagttcgagaactgctgtggcctgcgggaaggagctgtccttaccctgctgagtgacatcgcatcggctcttagataccttcacgaaaacagaatcatccatcgagacctgaagccagaaaacatcgttctgcagcaaggagagaaaagattaatacacaaaattattgatctaggatatgccaaggagctggatcagggcgaactgtgcacggagtttgtggggactctgcaatacctggcgccagagcttctggagcagcagaagtacaccgtgaccgttgactactggagcttcggcaccctggccttcgagtgcatcactggcttccggcccttcctccctaactggcagcctgtgcagtggcactccaaagtccggcagaagagcgaagtggacatcgttgttagtgaagacttgaatggagcagtgaagttttcaagttcgctacccttccccaataatcttaacagtgtcttggctgaacggctggagaagtggctgcagctgatgcttatgtggcaccctcggcaaaggggcacggatccccagtatggccccaacggctgcttcagagccctggatgacatcttgaacttgaagctggttcatgtcttgaacatggtcacaggcaccgttcacacataccccgtgacggaggatgagagtctgcagagcttaaaaaccagaatccaggaagacacggggatcctggagacagaccaggagctgctgcaagaggcagggctggtgctgctccctgacaagcctgctactcagtgcatctcagacagcaagacaaacgagggcctcacgttggacatggatcttgtttttctctttgacaacagtaaaatcaactatgagactcagatcaccccccgaccccaaccggaaagtgtcagctgtatccttcaggagcccaagcggaacctctccttcttccagctgaggaaagtgtggggccaagtctggcacagcatccagacgctgaaggaagactgtaaccggctgcagcagggacagcgagcagccatgatgagtctcctccggaataacagctgcctctctaagatgaagaacgccatggcctccacggcccagcagctcaaggccaagctggacttcttcaaaaccagcatccagatcgacctggagaagtataaagagcagaccgagtttgggatcacctcagataaattgctgctggcttggcgggagatggagcaggctgtggagcagtgtgggcgggagaatgacgtgaagcatctagtagagcggatgatggcactgcagactgacattgtggacctgcagaggagcccgatgggtcggaagcaggggggcaccctggatgacctagaggaacaagcgagggagctctaccgaagactcagggagaagccaagagaccaaaggacagaaggtgacagccaggagatggtacggctgctgcttcaggcaatccaaagctttgagaagaaagttcgggtgatttatacacagctcagtaagaccgtggtttgtaagcagaaggcactggagttgctgcccaaggtagaagaggtagtgagccttatgaacgaggacgagaggaccgtggtccggcttcaggagaagcggcagaaggaactctggaacctcctgaagatcgcctgtagcaaagtccgaggtcccgtgagtggaagcccagacagcatgaatgtgtctcgactcagtcaccctggtcagctaatgtcccagccttccagtgcctgtgacagcttacctgaatcagacaagaaaagtgaagaactggtggccgaagcccacgccctctgctcccggctagaaagtgcgctgcaggacactgtgaaggagcaagacagaagcttcacgactctagactggagctggttacagatggaggatgaagaaaggtgtagcctggagcaggcctgtgac

SEQ ID NO: 7 - DNA, 484 bp, Homo sapiens
  source 1..484: mol_type = genomic DNA
gagaacagtgaagtaggagcagccgtaagtccgggcagggtcctgtccataaaaggcttttcccgggccggctccccgccggcagcgtgccccgccccggcccgctccatctccaaagcatgcagagaatgtctcggcagccccggtagactgctccaacttggtgtctttccccaaatatggagcctgtgtggagtcactgggggagccgggggtggggagcggagccggcttcctctagcagggagggggccgaggagcgagccagtgggggaggctgacatcaccacggcggcagccctttaaacccctcacccagccagcgccccatcctgtctgtccgaacccagacacaagtcttcactccttcctgcgagccctgaggaagccttgtgagtgcattggctggggcttggagggaagttgggctggagctggacaggagcagtgggtgcatttcaggcaggctctcctgaggtcccag

SEQ ID NO: 8 - DNA, 510 bp, Mus musculus
  source 1..510: mol_type = genomic DNA
ctgcagtcaagactagttcccaccaactcgattttaaagccttgcaagaaggtggcttgtttgtcccttgcaggttcctttgctcgggccaaactctagaatgcctccccctttctttctcattgaagagcagacccaagtccgggtaacaaggaagggtttcagggtcctgcccataaaaggtttttcccggccgccctcagcaccgccccgccccgacccccgcagcatctccaaagcatgcagagaatgtctccggctgcccccgacagactgctccaacttggtgtctttccccaaatatggagcctgtgtggagtgagtggggcggcccggggtggtgagccaagcagacttccatgggcagggaggggcgccacggggcggcagaggggtgacatcactgcctaggcggcctttaaacccctcacccagccggcgccccggcccgtctgccccagcccagacaccgaagctactctccttccagtccacaaacgaccaagcctt

SEQ ID NO: 9 - DNA, 23 bp, synthetic construct
  source 1..23: mol_type = other DNA; note = primer
gcggtctggcagtaaaaactatc

SEQ ID NO: 10 - DNA, 23 bp, synthetic construct
  source 1..23: mol_type = other DNA; note = primer
gtgaaacagcattgctgtcactt

SEQ ID NO: 11 - DNA, 6668 bp, synthetic construct
  source 1..6668: mol_type = other DNA; note = pAAV-SM22alpha-mIKKbeta-CA-WPRE
cctgcaggcagctgcgcgctcgctcgctcactgaggccgcccgggcaaagcccgggcgtcgggcgacctttggtcgcccggcctcagtgagcgagcgagcgcgcagagagggagtggccaactccatcactaggggttcctgcggccgcacgcgtctgcagtcaagactagttcccaccaactcgattttaaagccttgcaagaaggtggcttgtttgtcccttgcaggttcctttgctcgggccaaactctagaatgcctccccctttctttctcattgaagagcagacccaagtccgggtaacaaggaagggtttcagggtcctgcccataaaaggtttttcccggccgccctcagcaccgccccgccccgacccccgcagcatctccaaagcatgcagagaatgtctccggctgcccccgacagactgctccaacttggtgtctttccccaaatatggagcctgtgtggagtgagtggggcggcccggggtggtgagccaagcagacttccatgggcagggaggggcgccacggggcggcagaggggtgacatcactgcctaggcggcctttaaacccctcacccagccggcgccccggcccgtctgccccagcccagacaccgaagctactctccttccagtccacaaacgaccaagccttgagctcggtaccgaattcgctagcgatccaccatggactacaaagacgatgacgacaagcttgcggccgcaatgagctggtcaccgtccctcccaacccagacatgtggagcctgggaaatgaaagaacgcctggggaccgggggatttggaaacgtcatccggtggcacaatcaggcgacaggtgaacagatcgccatcaagcaatgccgacaggagctcagcccaaagaacagagaccgctggtgcctcgaaatccagatcatgagaaggctgaaccatcccaatgtggtggctgcccgggatgtcccagaggggatgcagaacctggcacccaatgatttgccactgctggccatggagtactgccaaggaggagatctccgaagatacttgaaccagttcgagaactgctgtggcctgcgggaaggagctgtccttaccctgctgagtgacatcgcatcggctcttagataccttcacgaaaacagaatcatccatcgagacctgaagccagaaaacatcgttctgcagcaaggagagaaaagattaatacacaaaattattgatctaggatatgccaaggagctggatcagggcgaactgtgcacggagtttgtggggactctgcaatacctggcgccagagcttctggagcagcagaagtacaccgtgaccgttgactactggagcttcggcaccctggccttcgagtgcatcactggcttccggcccttcctccctaactggcagcctgtgcagtggcactccaaagtccggcagaagagcgaagtggacatcgttgttagtgaagacttgaatggagcagtgaagttttcaagttcgctacccttccccaataatcttaacagtgtcttggctgaacggctggagaagtggctgcagctgatgcttatgtggcaccctcggcaaaggggcacggatccccagtatggccccaacggctgcttcagagccctggatgacatcttgaacttgaagctggttcatgtcttgaacatggtcacaggcaccgttcacacataccccgtgacggaggatgagagtctgcagagcttaaaaaccagaatccaggaagacacggggatcctggagacagaccaggagctgctgcaagaggcagggctggtgctgctccctgacaagcctgctactcagtgcatctcagacagcaagacaaacgagggcctcacgttggacatggatcttgtttttctctttgacaacagtaaaatcaactatgagactcagatcaccccccgaccccaaccggaaagtgtcagctgtatccttcaggagcccaagcggaacctctccttcttccagctgaggaaagtgtggggccaagtctggcacagcatccagacgctgaaggaagactgtaaccggctgcagcagggacagcgagcagccatgatgagtctcctccggaataacagctgcctctctaagatgaagaacgccatggcctccacggcccagcagctcaaggccaagctggacttcttcaaaaccagcatccagatcgacctggagaagtataaagagcagaccgagtttgggatcacctcagataaattgctgctggcttggcgggagatggagcaggctgtggagcagtgtgggcgggagaatgacgtgaagcatctagtagagcggatgatggcactgcagactgacattgtggacctgcagaggagcccgatgggtcggaagcaggggggcaccctggatgacctagaggaacaagcgagggagctctaccgaagactcagggagaagccaagagaccaaaggacagaaggtgacagccaggagatggtacggctgctgcttcaggcaatccaaagctttgagaagaaagttcgggtgatttatacacagctcagtaagaccgtggtttgtaagcagaaggcactggagttgctgcccaaggtagaagaggtagtgagccttatgaacgaggacgagaggaccgtggtccggcttcaggagaagcggcagaaggaactctggaacctcctgaagatcgcctgtagcaaagtccgaggtcccgtgagtggaagcccagacagcatgaatgtgtctcgactcagtcaccctggtcagctaatgtcccagccttccagtgcctgtgacagcttacctgaatcagacaagaaaagtgaagaactggtggccgaagcccacgccctctgctcccggctagaaagtgcgctgcaggacactgtgaaggagcaagacagaagcttcacgactctagactggagctggttacagatggaggatgaagaaaggtgtagcctggagcaggcctgtgactgaatcggatccgtcgacaagctttctagaactagtctcgagcaattggggcccgtttaaacatcgataatcaacctctggattacaaaatttgtgaaagattgactggtattcttaactatgttgctccttttacgctatgtggatacgctgctttaatgcctttgtatcatgctattgcttcccgtatggctttcattttctcctccttgtataaatcctggttgctgtctctttatgaggagttgtggcccgttgtcaggcaacgtggcgtggtgtgcactgtgtttgctgacgcaacccccactggttggggcattgccaccacctgtcagctcctttccgggactttcgctttccccctccctattgccacggcggaactcatcgccgcctgccttgcccgctgctggacaggggctcggctgttgggcactgacaattccgtggtgttgtcggggaaatcatcgtcctttccttggctgctcgcctgtgttgccacctggattctgcgcgggacgtccttctgctacgtcccttcggccctcaatccagcggaccttccttcccgcggcctgctgccggctctgcggcctcttccgcgtcttcgccttcgccctcagacgagtcggatctccctttgggccgcctccccgcatcgaaacccgctgatcagcctcgactgtgccttctagttgccagccatctgttgtttgcccctcccccgtgccttccttgaccctggaaggtgccactcccactgtcctttcctaataaaatgaggaaattgcatcgcattgtctgagtaggtgtcattctattctggggggtggggtggggcaggacagcaagggggaggattgggaagacaatagcaggcatgctggggatgcggtgggctctatggcggaccgagcggccgcaggaacccctagtgatggagttggccactccctctctgcgcgctcgctcgctcactgaggccgggcgaccaaaggtcgcccgacgcccgggctttgcccgggcggcctcagtgagcgagcgagcgcgcagctgcctgcaggggcgcctgatgcggtattttctccttacgcatctgtgcggtatttcacaccgcatacgtcaaagcaaccatagtacgcgccctgtagcggcgcattaagcgcggcgggtgtggtggttacgcgcagcgtgaccgctacacttgccagcgccctagcgcccgctcctttcgctttcttcccttcctttctcgccacgttcgccggctttccccgtcaagctctaaatcgggggctccctttagggttccgatttagtgctttacggcacctcgaccccaaaaaacttgatttgggtgatggttcacgtagtgggccatcgccctgatagacggtttttcgccctttgacgttggagtccacgttctttaatagtggactcttgttccaaactggaacaacactcaaccctatctcgggctattcttttgatttataagggattttgccgatttcggcctattggttaaaaaatgagctgatttaacaaaaatttaacgcgaattttaacaaaatattaacgtttacaattttatggtgcactctcagtacaatctgctctgatgccgcatagttaagccagccccgacacccgccaacacccgctgacgcgccctgacgggcttgtctgctcccggcatccgcttacagacaagctgtgaccgtctccgggagctgcatgtgtcagaggttttcaccgtcatcaccgaaacgcgcgagacgaaagggcctcgtgatacgcctatttttataggttaatgtcatgataataatggtttcttagacgtcaggtggcacttttcggggaaatgtgcgcggaacccctatttgtttatttttctaaatacattcaaatatgtatccgctcatgagacaataaccctgataaatgcttcaataatattgaaaaaggaagagtatgagtattcaacatttccgtgtcgcccttattcccttttttgcggcattttgccttcctgtttttgctcacccagaaacgctggtgaaagtaaaagatgctgaagatcagttgggtgcacgagtgggttacatcgaactggatctcaacagcggtaagatccttgagagttttcgccccgaagaacgttttccaatgatgagcacttttaaagttctgctatgtggcgcggtattatcccgtattgacgccgggcaagagcaactcggtcgccgcatacactattctcagaatgacttggttgagtactcaccagtcacagaaaagcatcttacggatggcatgacagtaagagaattatgcagtgctgccataaccatgagtgataacactgcggccaacttacttctgacaacgatcggaggaccgaaggagctaaccgcttttttgcacaacatgggggatcatgtaactcgccttgatcgttgggaaccggagctgaatgaagccataccaaacgacgagcgtgacaccacgatgcctgtagcaatggcaacaacgttgcgcaaactattaactggcgaactacttactctagcttcccggcaacaattaatagactggatggaggcggataaagttgcaggaccacttctgcgctcggcccttccggctggctggtttattgctgataaatctggagccggtgagcgtgggtctcgcggtatcattgcagcactggggccagatggtaagccctcccgtatcgtagttatctacacgacggggagtcaggcaactatggatgaacgaaatagacagatcgctgagataggtgcctcactgattaagcattggtaactgtcagaccaagtttactcatatatactttagattgatttaaaacttcatttttaatttaaaaggatctaggtgaagatcctttttgataatctcatgaccaaaatcccttaacgtgagttttcgttccactgagcgtcagaccccgtagaaaagatcaaaggatcttcttgagatcctttttttctgcgcgtaatctgctgcttgcaaacaaaaaaaccaccgctaccagcggtggtttgtttgccggatcaagagctaccaactctttttccgaaggtaactggcttcagcagagcgcagataccaaatactgtccttctagtgtagccgtagttaggccaccacttcaagaactctgtagcaccgcctacatacctcgctctgctaatcctgttaccagtggctgctgccagtggcgataagtcgtgtcttaccgggttggactcaagacgatagttaccggataaggcgcagcggtcgggctgaacggggggttcgtgcacacagcccagcttggagcgaacgacctacaccgaactgagatacctacagcgtgagctatgagaaagcgccacgcttcccgaagggagaaaggcggacaggtatccggtaagcggcagggtcggaacaggagagcgcacgagggagcttccagggggaaacgcctggtatctttatagtcctgtcgggtttcgccacctctgacttgagcgtcgatttttgtgatgctcgtcaggggggcggagcctatggaaaaacgccagcaacgcggcctttttacggttcctggccttttgctggccttttgctcacatgt